European Patent Specification EP 4 000 629 B1, published November 5, 2025. Title: Compositions for Diagnosis, Prevention or Treatment of Fatty Liver Disease. Applicant: HysensBio Seoul National University & R & DB Foundation. Application EP. The sequence listing filed with the application follows.

SEQUENCE LISTING (10 sequences)

SEQ ID NO: 1 - DNA, 20 bp, Unknown
  mSREBF1
gcagtctgctttggaacctc

SEQ ID NO: 2 - DNA, 20 bp, Unknown
  mSREBF1
cctcctgtgtacttgcccat

SEQ ID NO: 3 - DNA, 22 bp, Unknown
  hSREBF1
tgtccacaaaagcaaatctctg

SEQ ID NO: 4 - DNA, 22 bp, Unknown
  hSREBF1
agtgtgtcctccacctcagtct

SEQ ID NO: 5 - DNA, 22 bp, Unknown
  hCPNE7
gtcttcacggtggactactact

SEQ ID NO: 6 - DNA, 21 bp, Unknown
  hCPNE7
atgcgtgtcgtacacctcaaa

SEQ ID NO: 7 - DNA, 21 bp, Unknown
  mGapdh
aggtcggtgtgaacggatttg

SEQ ID NO: 8 - DNA, 23 bp, Unknown
  mGapdh
tgtagaccatgtagttgaggtca

SEQ ID NO: 9 - DNA, 21 bp, Unknown
  hGAPDH
agggctgcttttaactctggt

SEQ ID NO: 10 - DNA, 21 bp, Unknown
  hGAPDH
ccccacttgattttggaggga